European Patent Application EP 4 570 316 A2, published June 18, 2025. Title: ANTAGONISTS OF THE COMPLEMENT SYSTEM FOR USE IN METHODS OF TREATING PARAPROTEINEMIC NEUROPATHIES. Applicant: ARGENX BV. Application EP. The sequence listing filed with the application follows.

SEQUENCE LISTING (31 sequences)

SEQ ID NO: 1 - protein, 752 aa, homo sapiens
MGPLMVLFCLLFLYPGLADSAPSCPQNVNISGGTFTLSHGWAPGSLLTYSCPQGLYPSPASRLCKSSGQWQTPGATRSLSKAVCKPVRCPAPVSFENGIYTPRLGSYPVGGNVSFECEDGFILRGSPVRQCRPNGMWDGETAVCDNGAGHCPNPGISLGAVRTGFRFGHGDKVRYRCSSNLVLTGSSERECQGNGVWSGTEPICRQPYSYDFPEDVAPALGTSFSHMLGATNPTQKTKESLGRKIQIQRSGHLNLYLLLDCSQSVSENDFLIFKESASLMVDRIFSFEINVSVAIITFASEPKVLMSVLNDNSRDMTEVISSLENANYKDHENGTGTNTYAALNSVYLMMNNQMRLLGMETMAWQEIRHAIILLTDGKSNMGGSPKTAVDHIREILNINQKRNDYLDIYAIGVGKLDVDWRELNELGSKKDGERHAFILQDTKALHQVFEHMLDVSKLTDTICGVGNMSANASDQERTPWHVTIKPKSQETCRGALISDQWVLTAAHCFRDGNDHSLWRVNVGDPKSQWGKEFLIEKAVISPGFDVFAKKNQGILEFYGDDIALLKLAQKVKMSTHARPICLPCTMEANLALRRPQGSTCRDHENELLNKQSVPAHFVALNGSKLNINLKMGVEWTSCAEVVSQEKTMFPNLTDVREVVTDQFLCSGTQEDESPCKGESGGAVFLERRFRFFQVGLVSWGLYNPCLGSADKNSRKRAPRSKVPPPRDFHINLFRMQPWLRQHLGDVLNFLPL

SEQ ID NO: 2 - protein, 9 aa, synthetic construct
EDDHDAFAY

SEQ ID NO: 3 - protein, 17 aa, synthetic construct
DINPNYESTGYNQKFKG

SEQ ID NO: 4 - protein, 5 aa, synthetic construct
DYNMD

SEQ ID NO: 5 - protein, 9 aa, synthetic construct
QHSRELPYT

SEQ ID NO: 6 - protein, 7 aa, synthetic construct
LASNLKS

SEQ ID NO: 7 - protein, 15 aa, synthetic construct
RASKSVRTSGYNYMH

SEQ ID NO: 8 - protein, 118 aa, synthetic construct
EVQLVQSGAEVKKPGASVKVSCKASGYTFTDYNMDWVRQATGQGLEWIGDINPNYESTGYNQKFKGRATMTVDKSISTAYMELSSLRSEDTAVYYCAREDDHDAFAYWGQGTLVTVSS

SEQ ID NO: 9 - protein, 111 aa, synthetic construct
DNVLTQSPDSLAVSLGERATISCRASKSVRTSGYNYMHWYQQKPGQPPKLLIYLASNLKSGVPDRFSGSGSGTDFTLTISSLQAEDAATYYCQHSRELPYTFGQGTKLEIK

SEQ ID NO: 10 - protein, 330 aa, homo sapiens [sequence omitted]

SEQ ID NO: 11 - protein, 329 aa, homo sapiens
ASTKGPSVFPLAPSSKSTSGGTAALGCLVKDYFPEPVTVSWNSGALTSGVHTFPAVLQSSGLYSLSSVVTVPSSSLGTQTYICNVNHKPSNTKVDKKVEPKSCDKTHTCPPCPAPEAAGGPSVFLFPPKPKDTLMISRTPEVTCVVVDVSHEDPEVKFNWYVDGVEVHNAKTKPREEQYNSTYRVVSVLTVLHQDWLNGKEYKCKVSNKALPAPIEKTISKAKGQPREPQVYTLPPSRDELTKNQVSLTCLVKGFYPSDIAVEWESNGQPENNYKTTPPVLDSDGSFFLYSKLTVDKSRWQQGNVFSCSVMHEALKFHYTQKSLSLSPG

SEQ ID NO: 12 - protein, 327 aa, homo sapiens
ASTKGPSVFPLAPCSRSTSESTAALGCLVKDYFPEPVTVSWNSGALTSGVHTFPAVLQSSGLYSLSSVVTVPSSSLGTKTYTCNVDHKPSNTKVDKRVESKYGPPCPSCPAPEFLGGPSVFLFPPKPKDTLMISRTPEVTCVVVDVSQEDPEVQFNWYVDGVEVHNAKTKPREEQFNSTYRVVSVLTVLHQDWLNGKEYKCKVSNKGLPSSIEKTISKAKGQPREPQVYTLPPSQEEMTKNQVSLTCLVKGFYPSDIAVEWESNGQPENNYKTTPPVLDSDGSFFLYSRLTVDKSRWQEGNVFSCSVMHEALHNHYTQKSLSLSLGK

SEQ ID NO: 13 - protein, 327 aa, homo sapiens
ASTKGPSVFPLAPCSRSTSESTAALGCLVKDYFPEPVTVSWNSGALTSGVHTFPAVLQSSGLYSLSSVVTVPSSSLGTKTYTCNVDHKPSNTKVDKRVESKYGPPCPPCPAPEFLGGPSVFLFPPKPKDTLMISRTPEVTCVVVDVSQEDPEVQFNWYVDGVEVHNAKTKPREEQFNSTYRVVSVLTVLHQDWLNGKEYKCKVSNKGLPSSIEKTISKAKGQPREPQVYTLPPSQEEMTKNQVSLTCLVKGFYPSDIAVEWESNGQPENNYKTTPPVLDSDGSFFLYSRLTVDKSRWQEGNVFSCSVMHEALHNHYTQKSLSLSPGK

SEQ ID NO: 14 - protein, 327 aa, homo sapiens
ASTKGPSVFPLAPCSRSTSESTAALGCLVKDYFPEPVTVSWNSGALTSGVHTFPAVLQSSGLYSLSSVVTVPSSSLGTKTYTCNVDHKPSNTKVDKRVESKYGPPCPPCPAPEFLGGPSVFLFPPKPKDTLMISRTPEVTCVVVDVSQEDPEVQFNWYVDGVEVHNAKTKPREEQFNSTYRVVSVLTVLHQDWLNGKEYKCKVSNKGLPSSIEKTISKAKGQPREPQVYTLPPSQEEMTKNQVSLTCLVKGFYPSDIAVEWESNGQPENNYKTTPPVLDSDGSFFLYSRLTVDKSRWQEGNVFSCSVMHEALKFHYTQKSLSLSPGK

SEQ ID NO: 15 - protein, 448 aa, synthetic construct
EVQLVQSGAEVKKPGASVKVSCKASGYTFTDYNMDWVRQATGQGLEWIGDINPNYESTGYNQKFKGRATMTVDKSISTAYMELSSLRSEDTAVYYCAREDDHDAFAYWGQGTLVTVSSASTKGPSVFPLAPSSKSTSGGTAALGCLVKDYFPEPVTVSWNSGALTSGVHTFPAVLQSSGLYSLSSVVTVPSSSLGTQTYICNVNHKPSNTKVDKKVEPKSCDKTHTCPPCPAPELLGGPSVFLFPPKPKDTLMISRTPEVTCVVVDVSHEDPEVKFNWYVDGVEVHNAKTKPREEQYNSTYRVVSVLTVLHQDWLNGKEYKCKVSNKALPAPIEKTISKAKGQPREPQVYTLPPSRDELTKNQVSLTCLVKGFYPSDIAVEWESNGQPENNYKTTPPVLDSDGSFFLYSKLTVDKSRWQQGNVFSCSVMHEALHNHYTQKSLSLSPGK

SEQ ID NO: 16 - protein, 447 aa, synthetic construct
EVQLVQSGAEVKKPGASVKVSCKASGYTFTDYNMDWVRQATGQGLEWIGDINPNYESTGYNQKFKGRATMTVDKSISTAYMELSSLRSEDTAVYYCAREDDHDAFAYWGQGTLVTVSSASTKGPSVFPLAPSSKSTSGGTAALGCLVKDYFPEPVTVSWNSGALTSGVHTFPAVLQSSGLYSLSSVVTVPSSSLGTQTYICNVNHKPSNTKVDKKVEPKSCDKTHTCPPCPAPEAAGGPSVFLFPPKPKDTLMISRTPEVTCVVVDVSHEDPEVKFNWYVDGVEVHNAKTKPREEQYNSTYRVVSVLTVLHQDWLNGKEYKCKVSNKALPAPIEKTISKAKGQPREPQVYTLPPSRDELTKNQVSLTCLVKGFYPSDIAVEWESNGQPENNYKTTPPVLDSDGSFFLYSKLTVDKSRWQQGNVFSCSVMHEALKFHYTQKSLSLSPG

SEQ ID NO: 17 - protein, 445 aa, synthetic construct
EVQLVQSGAEVKKPGASVKVSCKASGYTFTDYNMDWVRQATGQGLEWIGDINPNYESTGYNQKFKGRATMTVDKSISTAYMELSSLRSEDTAVYYCAREDDHDAFAYWGQGTLVTVSSASTKGPSVFPLAPCSRSTSESTAALGCLVKDYFPEPVTVSWNSGALTSGVHTFPAVLQSSGLYSLSSVVTVPSSSLGTKTYTCNVDHKPSNTKVDKRVESKYGPPCPSCPAPEFLGGPSVFLFPPKPKDTLMISRTPEVTCVVVDVSQEDPEVQFNWYVDGVEVHNAKTKPREEQFNSTYRVVSVLTVLHQDWLNGKEYKCKVSNKGLPSSIEKTISKAKGQPREPQVYTLPPSQEEMTKNQVSLTCLVKGFYPSDIAVEWESNGQPENNYKTTPPVLDSDGSFFLYSRLTVDKSRWQEGNVFSCSVMHEALHNHYTQKSLSLSLGK

SEQ ID NO: 18 - protein, 445 aa, synthetic construct
EVQLVQSGAEVKKPGASVKVSCKASGYTFTDYNMDWVRQATGQGLEWIGDINPNYESTGYNQKFKGRATMTVDKSISTAYMELSSLRSEDTAVYYCAREDDHDAFAYWGQGTLVTVSSASTKGPSVFPLAPCSRSTSESTAALGCLVKDYFPEPVTVSWNSGALTSGVHTFPAVLQSSGLYSLSSVVTVPSSSLGTKTYTCNVDHKPSNTKVDKRVESKYGPPCPPCPAPEFLGGPSVFLFPPKPKDTLMISRTPEVTCVVVDVSQEDPEVQFNWYVDGVEVHNAKTKPREEQFNSTYRVVSVLTVLHQDWLNGKEYKCKVSNKGLPSSIEKTISKAKGQPREPQVYTLPPSQEEMTKNQVSLTCLVKGFYPSDIAVEWESNGQPENNYKTTPPVLDSDGSFFLYSRLTVDKSRWQEGNVFSCSVMHEALHNHYTQKSLSLSPGK

SEQ ID NO: 19 - protein, 445 aa, synthetic construct
EVQLVQSGAEVKKPGASVKVSCKASGYTFTDYNMDWVRQATGQGLEWIGDINPNYESTGYNQKFKGRATMTVDKSISTAYMELSSLRSEDTAVYYCAREDDHDAFAYWGQGTLVTVSSASTKGPSVFPLAPCSRSTSESTAALGCLVKDYFPEPVTVSWNSGALTSGVHTFPAVLQSSGLYSLSSVVTVPSSSLGTKTYTCNVDHKPSNTKVDKRVESKYGPPCPPCPAPEFLGGPSVFLFPPKPKDTLMISRTPEVTCVVVDVSQEDPEVQFNWYVDGVEVHNAKTKPREEQFNSTYRVVSVLTVLHQDWLNGKEYKCKVSNKGLPSSIEKTISKAKGQPREPQVYTLPPSQEEMTKNQVSLTCLVKGFYPSDIAVEWESNGQPENNYKTTPPVLDSDGSFFLYSRLTVDKSRWQEGNVFSCSVMHEALKFHYTQKSLSLSPGK

SEQ ID NO: 20 - protein, 218 aa, synthetic construct
DNVLTQSPDSLAVSLGERATISCRASKSVRTSGYNYMHWYQQKPGQPPKLLIYLASNLKSGVPDRFSGSGSGTDFTLTISSLQAEDAATYYCQHSRELPYTFGQGTKLEIKRTVAAPSVFIFPPSDEQLKSGTASVVCLLNNFYPREAKVQWKVDNALQSGNSQESVTEQDSKDSTYSLSSTLTLSKADYEKHKVYACEVTHQGLSSPVTKSFNRGEC

SEQ ID NO: 21 - protein, 10 aa, homo sapiens
EPKSCDKTHT

SEQ ID NO: 22 - protein, 5 aa, homo sapiens
CPPCP

SEQ ID NO: 23 - protein, 8 aa, homo sapiens
APELLGGP

SEQ ID NO: 24 - protein, 12 aa, homo sapiens
ELKTPLGDTTHT

SEQ ID NO: 25 - protein, 50 aa, homo sapiens
CPRCPEPKSCDTPPPCPRCPEPKSCDTPPPCPRCPEPKSCDTPPPCPRCP

SEQ ID NO: 26 - protein, 7 aa, homo sapiens
ESKYGPP

SEQ ID NO: 27 - protein, 5 aa, homo sapiens
CPSCP

SEQ ID NO: 28 - protein, 8 aa, homo sapiens
APEFLGGP

SEQ ID NO: 29 - skipped

SEQ ID NO: 30 - protein, 10 aa, homo sapiens
CCVECPPPCP

SEQ ID NO: 31 - protein, 7 aa, homo sapiens
APPVAGP